European Patent Application EP 4 768 588 A1, published July 1, 2026. Title: miR-204에 대한 올리고뉴클레오타이드, 및 이를 포함하는 골관절염 개선, 예방 또는 치료용 조성물. Applicant: 라이플렉스사이언스 주식회사. The sequence listing filed with the application follows.

SEQUENCE LISTING (56 sequences)

SEQ ID NO: 1 - DNA, 22 bp, synthetic construct
  source 1..22: mol_type = other DNA
  modified_base 1..6: mod_base = OTHER; note = LNA (locked nucleic acid) sugar modification at positions 1-6
  modified_base 1..22: mod_base = OTHER; note = nucleotides 1-22 have phosphorothioate internucleotide linkages
  modified_base 14: mod_base = OTHER; note = iMe-dC (5-methyl-deoxycytosine) modified nucleoside at position 14
aggcataggatgacaaagggaa

SEQ ID NO: 2 - DNA, 22 bp, synthetic construct
  source 1..22: mol_type = other DNA
  modified_base 1..6: mod_base = OTHER; note = LNA (locked nucleic acid) sugar modification at positions 1-6
  modified_base 14: mod_base = OTHER; note = iMe-dC (5-methyl-deoxycytosine) modified nucleoside at position 14
aggcataggatgacaaagggaa

SEQ ID NO: 3 - DNA, 22 bp, synthetic construct
  source 1..22: mol_type = other DNA
  modified_base 1..6: mod_base = OTHER; note = LNA (locked nucleic acid) sugar modification at positions 1-6
  modified_base 1..22: mod_base = OTHER; note = Nucleotides 1-22 have phosphorothioate internucleotide linkage
aggcataggatgagaaagggaa

SEQ ID NO: 4 - DNA, 22 bp, synthetic construct
  source 1..22: mol_type = other DNA
  modified_base 1..6: mod_base = OTHER; note = LNA (locked nucleic acid) sugar modification at positions 1-6
  modified_base 1..22: mod_base = OTHER; note = Nucleotides 1-22 have phosphorothioate internucleotide linkage
  modified_base 14: mod_base = OTHER; note = iMe-dC (5-methyl-deoxycytosine) modified nucleoside at position 14
aggcataggaagacaaagggaa

SEQ ID NO: 5 - DNA, 22 bp, synthetic construct
  source 1..22: mol_type = other DNA
  modified_base 1..6: mod_base = OTHER; note = LNA (locked nucleic acid) sugar modification at positions 1-6
  modified_base 1..22: mod_base = OTHER; note = Nucleotides 1-22 have phosphorothioate internucleotide linkage
  modified_base 14: mod_base = OTHER; note = iMe-dC (5-methyl-deoxycytosine) modified nucleoside at position 14
aggcatacgaagacaaagggaa

SEQ ID NO: 6 - DNA, 21 bp, synthetic construct
  source 1..21: mol_type = other DNA
  modified_base 1..6: mod_base = OTHER; note = LNA (locked nucleic acid) sugar modification at positions 1-6
  modified_base 1..21: mod_base = OTHER; note = Nucleotides 1-21 have phosphorothioate internucleotide linkage
  modified_base 14: mod_base = OTHER; note = iMe-dC (5-methyl-deoxycytosine) modified nucleoside at position 14
aggcataggatgacaaaggga

SEQ ID NO: 7 - DNA, 20 bp, synthetic construct
  source 1..20: mol_type = other DNA
  modified_base 1..6: mod_base = OTHER; note = LNA (locked nucleic acid) sugar modification at positions 1-6
  modified_base 1..20: mod_base = OTHER; note = Nucleotides 1-20 have phosphorothioate internucleotide linkage
  modified_base 14: mod_base = OTHER; note = iMe-dC (5-methyl-deoxycytosine) modified nucleoside at position 14
aggcataggatgacaaaggg

SEQ ID NO: 8 - DNA, 22 bp, synthetic construct
  source 1..22: mol_type = other DNA
  modified_base 1..3: mod_base = OTHER; note = LNA (locked nucleic acid) sugar modification at positions 1-3
  modified_base 5: mod_base = OTHER; note = LNA (locked nucleic acid) sugar modification at position 5
  modified_base 6: mod_base = OTHER; note = LNA (locked nucleic acid) sugar modification at position 6
  modified_base 1..22: mod_base = OTHER; note = Nucleotides 1-22 have phosphorothioate internucleotide linkage
  modified_base 4: mod_base = OTHER; note = iMe-dC (5-methyl-deoxycytosine) modified nucleoside at position 4
  modified_base 14: mod_base = OTHER; note = iMe-dC (5-methyl-deoxycytosine) modified nucleoside at position 14
aggcataggatgacaaagggaa

SEQ ID NO: 9 - DNA, 22 bp, synthetic construct
  source 1..22: mol_type = other DNA
  modified_base 1..4: mod_base = OTHER; note = LNA (locked nucleic acid) sugar modification at positions 1-4
  modified_base 6: mod_base = OTHER; note = LNA (locked nucleic acid) sugar modification at position 6
  modified_base 1..22: mod_base = OTHER; note = Nucleotides 1-22 have phosphorothioate internucleotide linkage
  modified_base 14: mod_base = OTHER; note = iMe-dC (5-methyl-deoxycytosine) modified nucleoside at position 14
aggcataggatgacaaagggaa

SEQ ID NO: 10 - DNA, 22 bp, synthetic construct
  source 1..22: mol_type = other DNA
  modified_base 1..5: mod_base = OTHER; note = LNA (locked nucleic acid) sugar modification at positions 1-5
  modified_base 1..22: mod_base = OTHER; note = Nucleotides 1-22 have phosphorothioate internucleotide linkage
  modified_base 14: mod_base = OTHER; note = iMe-dC (5-methyl-deoxycytosine) modified nucleoside at position 14
aggcataggatgacaaagggaa

SEQ ID NO: 11 - DNA, 22 bp, synthetic construct
  source 1..22: mol_type = other DNA
  modified_base 1..3: mod_base = OTHER; note = LNA (locked nucleic acid) sugar modification at positions 1-3
  modified_base 6: mod_base = OTHER; note = LNA (locked nucleic acid) sugar modification at position 6
  modified_base 1..22: mod_base = OTHER; note = Nucleotides 1-22 have phosphorothioate internucleotide linkage
  modified_base 4: mod_base = OTHER; note = iMe-dC (5-methyl-deoxycytosine) modified nucleoside at position 4
  modified_base 14: mod_base = OTHER; note = iMe-dC (5-methyl-deoxycytosine) modified nucleoside at position 14
aggcataggatgacaaagggaa

SEQ ID NO: 12 - DNA, 22 bp, synthetic construct
  source 1..22: mol_type = other DNA
  modified_base 1..4: mod_base = OTHER; note = LNA (locked nucleic acid) sugar modification at positions 1-4
  modified_base 1..22: mod_base = OTHER; note = Nucleotides 1-22 have phosphorothioate internucleotide linkage
  modified_base 14: mod_base = OTHER; note = iMe-dC (5-methyl-deoxycytosine) modified nucleoside at position 14
aggcataggatgacaaagggaa

SEQ ID NO: 13 - DNA, 22 bp, synthetic construct
  source 1..22: mol_type = other DNA
  modified_base 1..3: mod_base = OTHER; note = LNA (locked nucleic acid) sugar modification at positions 1-3
  modified_base 1..22: mod_base = OTHER; note = Nucleotides 1-22 have phosphorothioate internucleotide linkage
  modified_base 5: mod_base = OTHER; note = LNA (locked nucleic acid) sugar modification at position 5
  modified_base 4: mod_base = OTHER; note = iMe-dC (5-methyl-deoxycytosine) modified nucleoside at position 4
  modified_base 14: mod_base = OTHER; note = iMe-dC (5-methyl-deoxycytosine) modified nucleoside at position 14
aggcataggatgacaaagggaa

SEQ ID NO: 14 - DNA, 22 bp, synthetic construct
  source 1..22: mol_type = other DNA
  modified_base 1..3: mod_base = OTHER; note = LNA (locked nucleic acid) sugar modification at positions 1-3
  modified_base 1..22: mod_base = OTHER; note = Nucleotides 1-22 have phosphorothioate internucleotide linkage
  modified_base 4: mod_base = OTHER; note = iMe-dC (5-methyl-deoxycytosine) modified nucleoside at position 4
  modified_base 14: mod_base = OTHER; note = iMe-dC (5-methyl-deoxycytosine) modified nucleoside at position 14
aggcataggatgacaaagggaa

SEQ ID NO: 15 - DNA, 22 bp, synthetic construct
  source 1..22: mol_type = other DNA
  modified_base 1: mod_base = OTHER; note = LNA (locked nucleic acid) sugar modification at position 1
  modified_base 1..22: mod_base = OTHER; note = Nucleotides 1-22 have phosphorothioate internucleotide linkage
  modified_base 4: mod_base = OTHER; note = iMe-dC (5-methyl-deoxycytosine) modified nucleoside at position 4
  modified_base 14: mod_base = OTHER; note = iMe-dC (5-methyl-deoxycytosine) modified nucleoside at position 14
aggcataggatgacaaagggaa

SEQ ID NO: 16 - DNA, 22 bp, synthetic construct
  source 1..22: mol_type = other DNA
  modified_base 1..2: mod_base = OTHER; note = LNA (locked nucleic acid) sugar modification at positions 1-2
  modified_base 1..22: mod_base = OTHER; note = Nucleotides 1-22 have phosphorothioate internucleotide linkage
  modified_base 4: mod_base = OTHER; note = iMe-dC (5-methyl-deoxycytosine) modified nucleoside at position 4
  modified_base 14: mod_base = OTHER; note = iMe-dC (5-methyl-deoxycytosine) modified nucleoside at position 14
aggcataggatgacaaagggaa

SEQ ID NO: 17 - DNA, 22 bp, synthetic construct
  source 1..22: mol_type = other DNA
  modified_base 22: mod_base = OTHER; note = LNA (locked nucleic acid) sugar modification at position 22
  modified_base 1..22: mod_base = OTHER; note = Nucleotides 1-22 have phosphorothioate internucleotide linkage
  modified_base 4: mod_base = OTHER; note = iMe-dC (5-methyl-deoxycytosine) modified nucleoside at position 4
  modified_base 14: mod_base = OTHER; note = iMe-dC (5-methyl-deoxycytosine) modified nucleoside at position 14
aggcataggatgacaaagggaa

SEQ ID NO: 18 - DNA, 22 bp, synthetic construct
  source 1..22: mol_type = other DNA
  modified_base 21..22: mod_base = OTHER; note = LNA (locked nucleic acid) sugar modification at positions 21-22
  modified_base 1..22: mod_base = OTHER; note = Nucleotides 1-22 have phosphorothioate internucleotide linkage
  modified_base 4: mod_base = OTHER; note = iMe-dC (5-methyl-deoxycytosine) modified nucleoside at position 4
  modified_base 14: mod_base = OTHER; note = iMe-dC (5-methyl-deoxycytosine) modified nucleoside at position 14
aggcataggatgacaaagggaa

SEQ ID NO: 19 - DNA, 22 bp, synthetic construct
  source 1..22: mol_type = other DNA
  modified_base 19..22: mod_base = OTHER; note = LNA (locked nucleic acid) sugar modification at positions 19-22
  modified_base 1..22: mod_base = OTHER; note = Nucleotides 1-22 have phosphorothioate internucleotide linkage
  modified_base 4: mod_base = OTHER; note = iMe-dC (5-methyl-deoxycytosine) modified nucleoside at position 4
  modified_base 14: mod_base = OTHER; note = iMe-dC (5-methyl-deoxycytosine) modified nucleoside at position 14
aggcataggatgacaaagggaa

SEQ ID NO: 20 - DNA, 22 bp, synthetic construct
  source 1..22: mol_type = other DNA
  modified_base 17..22: mod_base = OTHER; note = LNA (locked nucleic acid) sugar modification at positions 17-22
  modified_base 1..22: mod_base = OTHER; note = Nucleotides 1-22 have phosphorothioate internucleotide linkage
  modified_base 4: mod_base = OTHER; note = iMe-dC (5-methyl-deoxycytosine) modified nucleoside at position 4
  modified_base 14: mod_base = OTHER; note = iMe-dC (5-methyl-deoxycytosine) modified nucleoside at position 14
aggcataggatgacaaagggaa

SEQ ID NO: 21 - DNA, 15 bp, synthetic construct
  source 1..15: mol_type = other DNA
  modified_base 1: mod_base = OTHER; note = LNA (locked nucleic acid) sugar modification at position 1
  modified_base 3: mod_base = OTHER; note = LNA (locked nucleic acid) sugar modification at position 3
  modified_base 6..7: mod_base = OTHER; note = LNA (locked nucleic acid) sugar modification at positions 6-7
  modified_base 10: mod_base = OTHER; note = LNA (locked nucleic acid) sugar modification at position 10
  modified_base 12: mod_base = OTHER; note = LNA (locked nucleic acid) sugar modification at position 12
  modified_base 15: mod_base = OTHER; note = LNA (locked nucleic acid) sugar modification at position 15
  modified_base 1..15: mod_base = OTHER; note = Nucleotides 1-15 have phosphorothioate internucleotide linkage
aggatgacaaaggga

SEQ ID NO: 22 - DNA, 18 bp, synthetic construct
  source 1..18: mol_type = other DNA
  modified_base 1: mod_base = OTHER; note = LNA (locked nucleic acid) sugar modification at position 1
  modified_base 4: mod_base = OTHER; note = LNA (locked nucleic acid) sugar modification at position 4
  modified_base 8: mod_base = OTHER; note = LNA (locked nucleic acid) sugar modification at position 8
  modified_base 11: mod_base = OTHER; note = LNA (locked nucleic acid) sugar modification at position 11
  modified_base 15: mod_base = OTHER; note = LNA (locked nucleic acid) sugar modification at position 15
  modified_base 18: mod_base = OTHER; note = LNA (locked nucleic acid) sugar modification at position 18
  modified_base 1..18: mod_base = OTHER; note = Nucleotides 1-18 have phosphorothioate internucleotide linkage
cataggatgacaaaggga

SEQ ID NO: 23 - DNA, 22 bp, synthetic construct
  source 1..22: mol_type = other DNA
  modified_base 1..15: mod_base = OTHER; note = LNA (locked nucleic acid) sugar modification at positions 1-15
  modified_base 1..22: mod_base = OTHER; note = Nucleotides 1-22 have phosphorothioate internucleotide linkage
aggcataggatgacaaagggaa

SEQ ID NO: 24 - DNA, 22 bp, synthetic construct
  source 1..22: mol_type = other DNA
  modified_base 1..19: mod_base = OTHER; note = LNA (locked nucleic acid) sugar modification at positions 1-19
  modified_base 1..22: mod_base = OTHER; note = Nucleotides 1-22 have phosphorothioate internucleotide linkage
aggcataggatgacaaagggaa

SEQ ID NO: 25 - DNA, 22 bp, synthetic construct
  source 1..22: mol_type = other DNA
  modified_base 1..22: mod_base = OTHER; note = LNA (locked nucleic acid) sugar modification at positions 1-22
  modified_base 1..22: mod_base = OTHER; note = Nucleotides 1-22 have phosphorothioate internucleotide linkage
aggcataggatgacaaagggaa

SEQ ID NO: 26 - DNA, 22 bp, synthetic construct
  source 1..22: mol_type = other DNA
  modified_base 1..3: mod_base = OTHER; note = LNA (locked nucleic acid) sugar modification at positions 1-3
  modified_base 5..6: mod_base = OTHER; note = LNA (locked nucleic acid) sugar modification at positions 5-6
  modified_base 1..22: mod_base = OTHER; note = Nucleotides 1-22 have phosphorothioate internucleotide linkage
  modified_base 4: mod_base = OTHER; note = MOE (2-O-methoxyethyl) sugar modification at position 4
  modified_base 14: mod_base = OTHER; note = iMe-dC (5-methyl-deoxycytosine) modified nucleoside at position 14
aggcataggatgagaaagggaa

SEQ ID NO: 27 - DNA, 22 bp, synthetic construct
  source 1..22: mol_type = other DNA
  modified_base 1..4: mod_base = OTHER; note = LNA (locked nucleic acid) sugar modification at positions 1-4
  modified_base 6: mod_base = OTHER; note = LNA (locked nucleic acid) sugar modification at position 6
  modified_base 5: mod_base = OTHER; note = MOE (2-O-methoxyethyl) sugar modification at position 5
  modified_base 1..22: mod_base = OTHER; note = Nucleotides 1-22 have phosphorothioate internucleotide linkage
  modified_base 14: mod_base = OTHER; note = iMe-dC (5-methyl-deoxycytosine) modified nucleoside at position 14
aggcataggatgagaaagggaa

SEQ ID NO: 28 - DNA, 22 bp, synthetic construct
  source 1..22: mol_type = other DNA
  modified_base 1..5: mod_base = OTHER; note = LNA (locked nucleic acid) sugar modification at positions 1-5
  modified_base 6: mod_base = OTHER; note = MOE (2-O-methoxyethyl) sugar modification at position 6
  modified_base 1..22: mod_base = OTHER; note = Nucleotides 1-22 have phosphorothioate internucleotide linkage
  modified_base 14: mod_base = OTHER; note = iMe-dC (5-methyl-deoxycytosine) modified nucleoside at position 14
aggcataggatgagaaagggaa

SEQ ID NO: 29 - DNA, 22 bp, synthetic construct
  source 1..22: mol_type = other DNA
  modified_base 1..3: mod_base = OTHER; note = LNA (locked nucleic acid) sugar modification at positions 1-3
  modified_base 6: mod_base = OTHER; note = LNA (locked nucleic acid) sugar modification at position 6
  modified_base 4..5: mod_base = OTHER; note = MOE (2-O-methoxyethyl) sugar modification at positions 4-5
  modified_base 1..22: mod_base = OTHER; note = Nucleotides 1-22 have phosphorothioate internucleotide linkage
  modified_base 14: mod_base = OTHER; note = iMe-dC (5-methyl-deoxycytosine) modified nucleoside at position 14
aggcataggatgagaaagggaa

SEQ ID NO: 30 - DNA, 22 bp, synthetic construct
  source 1..22: mol_type = other DNA
  modified_base 1..22: mod_base = OTHER; note = Nucleotides 1-22 have phosphorothioate internucleotide linkage
  modified_base 5..6: mod_base = OTHER; note = MOE (2-O-methoxyethyl) sugar modification at positions 5-6
  modified_base 1..4: mod_base = OTHER; note = LNA (locked nucleic acid) sugar modification at positions 1-4
  modified_base 14: mod_base = OTHER; note = iMe-dC (5-methyl-deoxycytosine) modified nucleoside at position 14
aggcataggatgagaaagggaa

SEQ ID NO: 31 - DNA, 22 bp, synthetic construct
  source 1..22: mol_type = other DNA
  modified_base 1..3: mod_base = OTHER; note = LNA (locked nucleic acid) sugar modification at positions 1-3
  modified_base 5: mod_base = OTHER; note = LNA (locked nucleic acid) sugar modification at position 5
  modified_base 4: mod_base = OTHER; note = MOE (2-O-methoxyethyl) sugar modification at position 4
  modified_base 6: mod_base = OTHER; note = MOE (2-O-methoxyethyl) sugar modification at position 6
  modified_base 14: mod_base = OTHER; note = iMe-dC (5-methyl-deoxycytosine) modified nucleoside at position 14
aggcataggatgagaaagggaa

SEQ ID NO: 32 - DNA, 22 bp, synthetic construct
  source 1..22: mol_type = other DNA
  modified_base 1..3: mod_base = OTHER; note = LNA (locked nucleic acid) sugar modification at positions 1-3
  modified_base 4..6: mod_base = OTHER; note = MOE (2-O-methoxyethyl) sugar modification at positions 4-6
  modified_base 1..22: mod_base = OTHER; note = Nucleotides 1-22 have phosphorothioate internucleotide linkage
  modified_base 14: mod_base = OTHER; note = iMe-dC (5-methyl-deoxycytosine) modified nucleoside at position 14
aggcataggatgagaaagggaa

SEQ ID NO: 33 - DNA, 22 bp, synthetic construct
  source 1..22: mol_type = other DNA
  modified_base 1..3: mod_base = OTHER; note = LNA (locked nucleic acid) sugar modification at positions 1-3
  modified_base 5..6: mod_base = OTHER; note = LNA (locked nucleic acid) sugar modification at positions 5-6
  modified_base 4: mod_base = OTHER; note = OME (2'-O-Methyl) sugar modification at position 4
  modified_base 1..22: mod_base = OTHER; note = Nucleotides 1-22 have phosphorothioate internucleotide linkage
  modified_base 14: mod_base = OTHER; note = iMe-dC (5-methyl-deoxycytosine) modified nucleoside at position 14
aggcataggatgagaaagggaa

SEQ ID NO: 34 - DNA, 22 bp, synthetic construct
  source 1..22: mol_type = other DNA
  modified_base 1..4: mod_base = OTHER; note = LNA (locked nucleic acid) sugar modification at positions 1-4
  modified_base 6: mod_base = OTHER; note = LNA (locked nucleic acid) sugar modification at position 6
  modified_base 5: mod_base = OTHER; note = OME (2'-O-Methyl) sugar modification at position 5
  modified_base 1..22: mod_base = OTHER; note = Nucleotides 1-22 have phosphorothioate internucleotide linkage
  modified_base 14: mod_base = OTHER; note = iMe-dC (5-methyl-deoxycytosine) modified nucleoside at position 14
aggcataggatgagaaagggaa

SEQ ID NO: 35 - DNA, 22 bp, synthetic construct
  misc_feature 1..5: note = DNA
  misc_feature 6: note = RNA
  misc_feature 7..22: note = DNA
  source 1..22: mol_type = other DNA
  modified_base 1..5: mod_base = OTHER; note = LNA (locked nucleic acid) sugar modification at positions 1-5
  modified_base 6: mod_base = OTHER; note = OME (2'-O-Methyl) sugar modification at position 6
  modified_base 1..22: mod_base = OTHER; note = Nucleotides 1-22 have phosphorothioate internucleotide linkage
  modified_base 14: mod_base = OTHER; note = iMe-dC (5-methyl-deoxycytosine) modified nucleoside at position 14
aggcataggatgagaaagggaa

SEQ ID NO: 36 - DNA, 22 bp, synthetic construct
  source 1..22: mol_type = other DNA
  modified_base 1..3: mod_base = OTHER; note = LNA (locked nucleic acid) sugar modification at positions 1-3
  modified_base 6: mod_base = OTHER; note = LNA (locked nucleic acid) sugar modification at position 6
  modified_base 4..5: mod_base = OTHER; note = OME (2'-O-Methyl) sugar modification at positions 4-5
  modified_base 1..22: mod_base = OTHER; note = Nucleotides 1-22 have phosphorothioate internucleotide linkage
  modified_base 14: mod_base = OTHER; note = iMe-dC (5-methyl-deoxycytosine) modified nucleoside at position 14
aggcataggatgagaaagggaa

SEQ ID NO: 37 - DNA, 22 bp, synthetic construct
  misc_feature 1..5: note = DNA
  misc_feature 6: note = RNA
  misc_feature 7..22: note = DNA
  source 1..22: mol_type = other DNA
  modified_base 1..4: mod_base = OTHER; note = LNA (locked nucleic acid) sugar modification at positions 1-4
  modified_base 5..6: mod_base = OTHER; note = OME (2'-O-Methyl) sugar modification at positions 5-6
  modified_base 1..22: mod_base = OTHER; note = Nucleotides 1-22 have phosphorothioate internucleotide linkage
  modified_base 14: mod_base = OTHER; note = iMe-dC (5-methyl-deoxycytosine) modified nucleoside at position 14
aggcataggatgagaaagggaa

SEQ ID NO: 38 - DNA, 22 bp, synthetic construct
  misc_feature 1..5: note = DNA
  misc_feature 6: note = RNA
  misc_feature 7..22: note = DNA
  source 1..22: mol_type = other DNA
  modified_base 1..3: mod_base = OTHER; note = LNA (locked nucleic acid) sugar modification at positions 1-3
  modified_base 5: mod_base = OTHER; note = LNA (locked nucleic acid) sugar modification at position 5
  modified_base 4: mod_base = OTHER; note = OME (2'-O-Methyl) sugar modification at position 4
  modified_base 6: mod_base = OTHER; note = OME (2'-O-Methyl) sugar modification at position 6
  modified_base 1..22: mod_base = OTHER; note = Nucleotides 1-22 have phosphorothioate internucleotide linkage
  modified_base 14: mod_base = OTHER; note = iMe-dC (5-methyl-deoxycytosine) modified nucleoside at position 14
aggcataggatgagaaagggaa

SEQ ID NO: 39 - DNA, 22 bp, synthetic construct
  misc_feature 1..5: note = DNA
  misc_feature 6: note = RNA
  misc_feature 7..22: note = DNA
  source 1..22: mol_type = other DNA
  modified_base 1..3: mod_base = OTHER; note = LNA (locked nucleic acid) sugar modification at positions 1-3
  modified_base 4..6: mod_base = OTHER; note = OME (2'-O-Methyl) sugar modification at positions 4-6
  modified_base 1..22: mod_base = OTHER; note = Nucleotides 1-22 have phosphorothioate internucleotide linkage
  modified_base 14: mod_base = OTHER; note = iMe-dC (5-methyl-deoxycytosine) modified nucleoside at position 14
aggcataggatgagaaagggaa

SEQ ID NO: 40 - DNA, 22 bp, synthetic construct
  source 1..22: mol_type = other DNA
  modified_base 1..22: mod_base = OTHER; note = Nucleotides 1-22 have phosphorothioate internucleotide linkage
  modified_base 4: mod_base = OTHER; note = iMe-dC (5-methyl-deoxycytosine) modified nucleoside at position 4
  modified_base 14: mod_base = OTHER; note = iMe-dC (5-methyl-deoxycytosine) modified nucleoside at position 14
aggcataggatgacaaagggaa

SEQ ID NO: 41 - DNA, 21 bp, synthetic construct
  source 1..21: mol_type = other DNA
aacccaagaagagagcagatg

SEQ ID NO: 42 - DNA, 21 bp, synthetic construct
  source 1..21: mol_type = other DNA
agcctggagaatagtagatgc

SEQ ID NO: 43 - DNA, 22 bp, synthetic construct
  source 1..22: mol_type = other DNA
tggtcattctgcttttcaactc

SEQ ID NO: 44 - DNA, 20 bp, synthetic construct
  source 1..20: mol_type = other DNA
actcggtaatctcgcatcag

SEQ ID NO: 45 - DNA, 21 bp, synthetic construct
  source 1..21: mol_type = other DNA
caggacaagcagagaagagtc

SEQ ID NO: 46 - DNA, 20 bp, synthetic construct
  source 1..20: mol_type = other DNA
tcctccagggtaagatccgt

SEQ ID NO: 47 - DNA, 22 bp, synthetic construct
  source 1..22: mol_type = other DNA
gcgtggattatgtacaggtgtg

SEQ ID NO: 48 - DNA, 20 bp, synthetic construct
  source 1..20: mol_type = other DNA
gtctgctggttcagccatct

SEQ ID NO: 49 - DNA, 21 bp, synthetic construct
  source 1..21: mol_type = other DNA
atacaaagcctaagatgagcg

SEQ ID NO: 50 - DNA, 20 bp, synthetic construct
  source 1..20: mol_type = other DNA
gcaaatcaaaagtctgggga

SEQ ID NO: 51 - DNA, 22 bp, synthetic construct
  source 1..22: mol_type = other DNA
ggagacttcacagaggatacca

SEQ ID NO: 52 - DNA, 22 bp, synthetic construct
  source 1..22: mol_type = other DNA
tcatttccacgatttcccagag

SEQ ID NO: 53 - DNA, 20 bp, synthetic construct
  source 1..20: mol_type = other DNA
ttgatgggcctggaacagtc

SEQ ID NO: 54 - DNA, 20 bp, synthetic construct
  source 1..20: mol_type = other DNA
agtcctgagagatttgcgcc

SEQ ID NO: 55 - DNA, 22 bp, synthetic construct
  source 1..22: mol_type = other DNA
tgctcaccaactacagatttcc

SEQ ID NO: 56 - DNA, 21 bp, synthetic construct
  source 1..21: mol_type = other DNA
gctgctgtcaggacatcattg